European Patent Specification EP 3 888 667 B1, published October 25, 2023. Title: GLUCAGON ANALOGS AND METHODS OF USE THEREOF. Applicant: AMIDEBIO LLC. The sequence listing filed with the application follows.

SEQUENCE LISTING (30 sequences)

SEQ ID NO: 1 - protein, 29 aa, Artificial Sequence
  Description of Artificial Sequence: Synthetic peptide
HSQGTFTSDYSKYLDSRRAQDFVQELANT

SEQ ID NO: 2 - protein, 29 aa, Artificial Sequence
  Description of Artificial Sequence: Synthetic peptide
HSQGTFTSDYSKYLDSRRAQDFVQKLANT

SEQ ID NO: 3 - protein, 29 aa, Artificial Sequence
  Description of Artificial Sequence: Synthetic peptide
HSQGTFTSDYSKYLDSRRAQDFAQELANT

SEQ ID NO: 4 - protein, 29 aa, Artificial Sequence
  Description of Artificial Sequence: Synthetic peptide
HSQGTFTSDYSKYLDSRRAQDFAQKLANT

SEQ ID NO: 5 - protein, 29 aa, Artificial Sequence
  Description of Artificial Sequence: Synthetic peptide
HSQGTFTSDYSKYLDSRRAQDFVQDLANT

SEQ ID NO: 6 - protein, 29 aa, Artificial Sequence
  Description of Artificial Sequence: Synthetic peptide
HSQGTFTSDYSKYLDSRRAQDFVQHLANT

SEQ ID NO: 7 - protein, 29 aa, Artificial Sequence
  Description of Artificial Sequence: Synthetic peptide
HSQGTFTSDYSKYLDSRRAQDFVQDLADT

SEQ ID NO: 8 - protein, 29 aa, Artificial Sequence
  Description of Artificial Sequence: Synthetic peptide
HSQGTFTSDYSKYLDSRRAQDFVQDLAET

SEQ ID NO: 9 - protein, 29 aa, Artificial Sequence
  Description of Artificial Sequence: Synthetic peptide
HSQGTFTSDYSKYLDSRRAQDFVQKLENT

SEQ ID NO: 10 - protein, 29 aa, Artificial Sequence
  Description of Artificial Sequence: Synthetic peptide
HSQGTFTSDYSKYLDSRRAQDFVEKLENT

SEQ ID NO: 11 - protein, 29 aa, Artificial Sequence
  Description of Artificial Sequence: Synthetic peptide
HSQGTFTSDYSKYLDSRRAQDFVEKLEST

SEQ ID NO: 12 - protein, 29 aa, Artificial Sequence
  Description of Artificial Sequence: Synthetic peptide
HSQGTFTSDYSKYLDSRRAQDFVQKLLNT

SEQ ID NO: 13 - protein, 29 aa, Artificial Sequence
  Description of Artificial Sequence: Synthetic peptide
HSQGTFTSDYSKYLDSRRAQDFVQKLLST

SEQ ID NO: 14 - protein, 29 aa, Artificial Sequence
  Description of Artificial Sequence: Synthetic peptide
HSQGTFTSDYSKYLDSRRAQDFVEKLLST

SEQ ID NO: 15 - protein, 29 aa, Artificial Sequence
  Description of Artificial Sequence: Synthetic peptide
HSQGTFTSDYSKYLDSRRAQDFVEKLEKT

SEQ ID NO: 16 - protein, 29 aa, Artificial Sequence
  Description of Artificial Sequence: Synthetic peptide
HSQGTFTSDYSKYLDSRRAQDFVEKLANT

SEQ ID NO: 17 - protein, 29 aa, Artificial Sequence
  Description of Artificial Sequence: Synthetic peptide
HSQGTFTSDYSKYLDSRRAQDFVEKLAST

SEQ ID NO: 18 - protein, 29 aa, Artificial Sequence
  Description of Artificial Sequence: Synthetic peptide
HSQGTFTSDYSKYLDSRRAQDFVAKLANT

SEQ ID NO: 19 - protein, 29 aa, Artificial Sequence
  Description of Artificial Sequence: Synthetic peptide
HSQGTFTSDYSKYLDSRRAQDFVAKLAKT

SEQ ID NO: 20 - protein, 29 aa, Unknown
  Description of Unknown: Native glucagon sequence
HSQGTFTSDYSKYLDSRRAQDFVQWLMNT

SEQ ID NO: 21 - protein, 38 aa, Artificial Sequence
  Description of Artificial Sequence: Synthetic polypeptide
MKAIFVLKGSLDRDPEFPSDKPHHKKHHKKHHSSGSLE

SEQ ID NO: 22 - protein, 10 aa, Artificial Sequence
  Description of Artificial Sequence: Synthetic peptide
  MISC_FEATURE (1)..(10): This sequence may encompass 5-10 residues
KKKKKKKKKK

SEQ ID NO: 23 - protein, 10 aa, Artificial Sequence
  Description of Artificial Sequence: Synthetic peptide
  MISC_FEATURE (1)..(10): This sequence may encompass 5-10 residues
HHHHHHHHHH

SEQ ID NO: 24 - protein, 10 aa, Artificial Sequence
  Description of Artificial Sequence: Synthetic peptide
  MISC_FEATURE (1)..(10): This sequence may encompass 5-10 residues
EEEEEEEEEE

SEQ ID NO: 25 - protein, 10 aa, Artificial Sequence
  Description of Artificial Sequence: Synthetic peptide
  MISC_FEATURE (1)..(10): This sequence may encompass 5-10 residues
RRRRRRRRRR

SEQ ID NO: 26 - protein, 6 aa, Artificial Sequence
  Description of Artificial Sequence: Synthetic 6xHis tag
HHHHHH

SEQ ID NO: 27 - protein, 6 aa, Artificial Sequence
  Description of Artificial Sequence: Synthetic peptide
KKKKKK

SEQ ID NO: 28 - protein, 6 aa, Artificial Sequence
  Description of Artificial Sequence: Synthetic peptide
EEEEEE

SEQ ID NO: 29 - protein, 6 aa, Artificial Sequence
  Description of Artificial Sequence: Synthetic peptide
RRRRRR

SEQ ID NO: 30 - protein, 22 aa, Unknown
  Description of Unknown: Insulin sequence
FVNQHLCGSHLVEALYLVCGER